European Patent Application EP 4 276 106 A2, published November 15, 2023. Title: METHODS AND COMPOSITIONS FOR INDUCING AN IMMUNE RESPONSE USING CONSERVED ELEMENT CONSTRUCTS. Applicant: THE UNITED STATES OF AMERICA AS REPRESENTED BY THE SECRETARY OF THE DEPARTMENT OF HEALTH AND HUMAN SERVICES. Application EP, filed May 13, 2016. The sequence listing filed with the application follows.

SEQUENCE LISTING (89 sequences)

SEQ ID NO: 1 - protein, 11 aa, synthetic construct
  REGION 1..11: note = synthetic peptide construct
WVTVYYGVPVW

SEQ ID NO: 2 - protein, 14 aa, synthetic construct
  REGION 1..14: note = synthetic peptide construct
HNVWATHACVPTDP

SEQ ID NO: 3 - protein, 14 aa, synthetic construct
  REGION 1..14: note = synthetic peptide construct
HNIWATHACVPTDP

SEQ ID NO: 4 - protein, 21 aa, synthetic construct
  REGION 1..21: note = synthetic peptide construct
ISLWDQSLKPCVKLTPLCVTL

SEQ ID NO: 5 - protein, 21 aa, synthetic construct
  REGION 1..21: note = synthetic peptide construct
ISLWDESLKPCVKLTPLCVTL

SEQ ID NO: 6 - protein, 15 aa, synthetic construct
  REGION 1..15: note = synthetic peptide construct
FEPIPIHYCTPAGFA

SEQ ID NO: 7 - protein, 15 aa, synthetic construct
  REGION 1..15: note = synthetic peptide construct
FDPIPIHYCAPAGYA

SEQ ID NO: 8 - protein, 23 aa, synthetic construct
  REGION 1..23: note = synthetic peptide construct
VQCTHGIRPVVSTQLLLNGSLAE

SEQ ID NO: 9 - protein, 23 aa, synthetic construct
  REGION 1..23: note = synthetic peptide construct
VQCTHGIKPVVSTQLLLNGSLAE

SEQ ID NO: 10 - protein, 21 aa, synthetic construct
  REGION 1..21: note = synthetic peptide construct
SGGDPEIVMHSFNCGGEFFYC

SEQ ID NO: 11 - protein, 21 aa, synthetic construct
  REGION 1..21: note = synthetic peptide construct
AGGDLEITTHSFNCRGEFFYC

SEQ ID NO: 12 - protein, 13 aa, synthetic construct
  REGION 1..13: note = synthetic peptide construct
DNWRSELYKYKVV

SEQ ID NO: 13 - protein, 13 aa, synthetic construct
  REGION 1..13: note = synthetic peptide construct
NNWRSELYKYKVV

SEQ ID NO: 14 - protein, 12 aa, synthetic construct
  REGION 1..12: note = synthetic peptide construct
ARRRVVQREKRA

SEQ ID NO: 15 - protein, 12 aa, synthetic construct
  REGION 1..12: note = synthetic peptide construct
AKRRVVEREKRA

SEQ ID NO: 16 - protein, 14 aa, synthetic construct
  REGION 1..14: note = synthetic peptide construct
GFLGTAGSTMGAAS

SEQ ID NO: 17 - protein, 14 aa, synthetic construct
  REGION 1..14: note = synthetic peptide construct
GFLGAAGSTMGAAS

SEQ ID NO: 18 - protein, 43 aa, synthetic construct
  REGION 1..43: note = synthetic peptide construct
LTVQARLLLSGIVQQQNNLLRAIEAQQHLLQLTVWGIKQLQAR

SEQ ID NO: 19 - protein, 43 aa, synthetic construct
  REGION 1..43: note = synthetic peptide construct
LTVQARQLLSGIVQQQSNLLKAIEAQQHMLQLTVWGIKQLQTR

SEQ ID NO: 20 - protein, 20 aa, synthetic construct
  REGION 1..20: note = synthetic peptide construct
WLWYIKIFIMIVGGLVGLRI

SEQ ID NO: 21 - protein, 20 aa, synthetic construct
  REGION 1..20: note = synthetic peptide construct
WLWYIRIFIMIVGGLIGLRI

SEQ ID NO: 22 - protein, 13 aa, synthetic construct
  REGION 1..13: note = synthetic peptide construct
RVRKGYSPLSLQT

SEQ ID NO: 23 - protein, 13 aa, synthetic construct
  REGION 1..13: note = synthetic peptide construct
RVRQGYSPLSFQT

SEQ ID NO: 24 - protein, 253 aa, synthetic construct
  REGION 1..253: note = synthetic peptide construct
WVTVYYGVPVWAAVHNVWATHACVPTDPAAEISLWDQSLKPCVKLTPLCVTLGAKFEPIPIHYCTPAGFAGAKVQCTHGIRPVVSTQLLLNGSLAEAADSGGDPEIVMHSFNCGGEFFYCGAKDNWRSELYKYKVVAAKARRRVVQREKRAGAVGFLGTAGSTMGAASVAVLTVQARLLLSGIVQQQNNLLRAIEAQQHLLQLTVWGIKQLQARAADWLWYIKIFIMIVGGLVGLRIAAFRVRKGYSPLSLQT

SEQ ID NO: 25 - protein, 253 aa, synthetic construct
  REGION 1..253: note = synthetic peptide construct
WVTVYYGVPVWAAVHNIWATHACVPTDPAAEISLWDESLKPCVKLTPLCVTLGAKFDPIPIHYCAPAGYAGAKVQCTHGIKPVVSTQLLLNGSLAEAADAGGDLEITTHSFNCRGEFFYCGAKNNWRSELYKYKVVAAKAKRRVVEREKRAGAVGFLGAAGSTMGAASVAVLTVQARQLLSGIVQQQSNLLKAIEAQQHMLQLTVWGIKQLQTRAADWLWYIRIFIMIVGGLIGLRIAAFRVRQGYSPLSFQT

SEQ ID NO: 26 - protein, 12 aa, synthetic construct
  REGION 1..12: note = synthetic peptide construct
ISPRTLNAWVKV

SEQ ID NO: 27 - protein, 18 aa, synthetic construct
  REGION 1..18: note = synthetic peptide construct
VIPMFSALSEGATPQDLN

SEQ ID NO: 28 - protein, 24 aa, synthetic construct
  REGION 1..24: note = synthetic peptide construct
VGGHQAAMQMLKDTINEEAAEWDR

SEQ ID NO: 29 - protein, 19 aa, synthetic construct
  REGION 1..19: note = synthetic peptide construct
PRGSDIAGTTSTLQEQIGW

SEQ ID NO: 30 - protein, 20 aa, synthetic construct
  REGION 1..20: note = synthetic peptide construct
KRWIILGLNKIVRMYSPTSI

SEQ ID NO: 31 - protein, 14 aa, synthetic construct
  REGION 1..14: note = synthetic peptide construct
YVDRFYKTLRAEQA

SEQ ID NO: 32 - protein, 17 aa, synthetic construct
  REGION 1..17: note = synthetic peptide construct
LEEMMTACQGVGGPGHK

SEQ ID NO: 33 - protein, 12 aa, synthetic construct
  REGION 1..12: note = synthetic peptide construct
LSPRTLNAWVKV

SEQ ID NO: 34 - protein, 18 aa, synthetic construct
  REGION 1..18: note = synthetic peptide construct
VIPMFTALSEGATPQDLN

SEQ ID NO: 35 - protein, 24 aa, synthetic construct
  REGION 1..24: note = synthetic peptide construct
VGGHQAAMQMLKETINEEAAEWDR

SEQ ID NO: 36 - protein, 19 aa, synthetic construct
  REGION 1..19: note = synthetic peptide construct
PRGSDIAGTTSTLQEQIAW

SEQ ID NO: 37 - protein, 20 aa, synthetic construct
  REGION 1..20: note = synthetic peptide construct
KRWIILGLNKIVRMYSPVSI

SEQ ID NO: 38 - protein, 14 aa, synthetic construct
  REGION 1..14: note = synthetic peptide construct
YVDRFFKTLRAEQA

SEQ ID NO: 39 - protein, 17 aa, synthetic construct
  REGION 1..17: note = synthetic peptide construct
LEEMMTACQGVGGPSHK

SEQ ID NO: 40 - protein, 140 aa, synthetic construct
  REGION 1..140: note = synthetic peptide construct
VIPMFSALSEGATPQDLNAAVGGHQAAMQMLKDTINEEAAEWDRAAAEPRGSDIAGTTSTLQEQIGWAAAKRWIILGLNKIVRMYSPTSIAAKYVDRFYKTLRAEQAAGLEEMMTACQGVGGPGHKAAISPRTLNAWVKV

SEQ ID NO: 41 - protein, 140 aa, synthetic construct
  REGION 1..140: note = synthetic peptide construct
VIPMFTALSEGATPQDLNAAVGGHQAAMQMLKETINEEAAEWDRAAAEPRGSDIAGTTSTLQEQIAWAAAKRWIILGLNKIVRMYSPVSIAAKYVDRFFKTLRAEQAAGLEEMMTACQGVGGPSHKAALSPRTLNAWVKV

SEQ ID NO: 42 - protein, 157 aa, synthetic construct
  REGION 1..157: note = synthetic peptide construct
MWLQSLLLLGTVACSISVIPMFSALSEGATPQDLNAAVGGHQAAMQMLKDTINEEAAEWDRAAAEPRGSDIAGTTSTLQEQIGWAAAKRWIILGLNKIVRMYSPTSIAAKYVDRFYKTLRAEQAAGLEEMMTACQGVGGPGHKAAISPRTLNAWVKV

SEQ ID NO: 43 - protein, 157 aa, synthetic construct
  REGION 1..157: note = synthetic peptide construct
MWLQSLLLLGTVACSISVIPMFTALSEGATPQDLNAAVGGHQAAMQMLKETINEEAAEWDRAAAEPRGSDIAGTTSTLQEQIAWAAAKRWIILGLNKIVRMYSPVSIAAKYVDRFFKTLRAEQAAGLEEMMTACQGVGGPSHKAALSPRTLNAWVKV

SEQ ID NO: 44 - protein, 564 aa, synthetic construct
  REGION 1..564: note = synthetic peptide construct
MAPRSARRPLLLLLLLLLLGLMHCASAAMFMVKNGNGTACIMANFSAAFSVNYDTKSGPKNMTLDLPSDATVVLNRSSCGKENTSDPSLVIAFGRGHTLTLNFTRNATRYSVQLMSFVYNLSDTHLFPNASSKEIKTVESITDIRADIDKKYRCVSGTQVHMNNVTVTLHDATIQAYLSNSSFSRGETRCEQDRPSPTTAPPAPPSPSPSPVPKSPSVDKYNVSGTNGTCLLASMGLQLNLTYERKDNTTVTRLLNINPNKTSASGSCGAHLVTLELHSEGTTVLLFQFGMNASSSRFFLQGIQLNTILPDARDPAFKAANGSLRALQATVGNSYKCNAEEHVRVTKAFSVNIFKVWVQAFKVEGGQFGSVEECLLDENSLEDIVIPMFSALSEGATPQDLNAAVGGHQAAMQMLKDTINEEAAEWDRAAAEPRGSDIAGTTSTLQEQIGWAAAKRWIILGLNKIVRMYSPTSIAAKYVDRFYKTLRAEQAAGLEEMMTACQGVGGPGHKAAISPRTLNAWVKVGSEFTLIPIAVGGALAGLVLIVLIAYLVGRKRSHAGYQTI

SEQ ID NO: 45 - protein, 564 aa, synthetic construct
  REGION 1..564: note = synthetic peptide construct
MAPRSARRPLLLLLLLLLLGLMHCASAAMFMVKNGNGTACIMANFSAAFSVNYDTKSGPKNMTLDLPSDATVVLNRSSCGKENTSDPSLVIAFGRGHTLTLNFTRNATRYSVQLMSFVYNLSDTHLFPNASSKEIKTVESITDIRADIDKKYRCVSGTQVHMNNVTVTLHDATIQAYLSNSSFSRGETRCEQDRPSPTTAPPAPPSPSPSPVPKSPSVDKYNVSGTNGTCLLASMGLQLNLTYERKDNTTVTRLLNINPNKTSASGSCGAHLVTLELHSEGTTVLLFQFGMNASSSRFFLQGIQLNTILPDARDPAFKAANGSLRALQATVGNSYKCNAEEHVRVTKAFSVNIFKVWVQAFKVEGGQFGSVEECLLDENSLEDIVIPMFTALSEGATPQDLNAAVGGHQAAMQMLKETINEEAAEWDRAAAEPRGSDIAGTTSTLQEQIAWAAAKRWIILGLNKIVRMYSPVSIAAKYVDRFFKTLRAEQAAGLEEMMTACQGVGGPSHKAALSPRTLNAWVKVGSEFTLIPIAVGGALAGLVLIVLIAYLVGRKRSHAGYQTI

SEQ ID NO: 46 - protein, 157 aa, synthetic construct; identical to SEQ ID NO: 43
  REGION 1..157: note = synthetic peptide construct

SEQ ID NO: 47 - protein, 249 aa, synthetic construct
  REGION 1..249: note = synthetic peptide construct
MWKPMPSPSNMKASAALLCLLLTAAAFSPQGLAQPVGINTSTTCCYRFINKKIPKQRLESYRRTTSSHCPREAVIFKTKLDKEICADPTQKWVQDFMKHLDKKTQTPKLVIPMFSALSEGATPQDLNAAVGGHQAAMQMLKDTINEEAAEWDRAAAEPRGSDIAGTTSTLQEQIGWAAAKRWIILGLNKIVRMYSPTSIAAKYVDRFYKTLRAEQAAGLEEMMTACQGVGGPGHKAAISPRTLNAWVKV

SEQ ID NO: 48 - protein, 249 aa, synthetic construct
  REGION 1..249: note = synthetic peptide construct
MWKPMPSPSNMKASAALLCLLLTAAAFSPQGLAQPVGINTSTTCCYRFINKKIPKQRLESYRRTTSSHCPREAVIFKTKLDKEICADPTQKWVQDFMKHLDKKTQTPKLVIPMFTALSEGATPQDLNAAVGGHQAAMQMLKETINEEAAEWDRAAAEPRGSDIAGTTSTLQEQIAWAAAKRWIILGLNKIVRMYSPVSIAAKYVDRFFKTLRAEQAAGLEEMMTACQGVGGPSHKAALSPRTLNAWVKV

SEQ ID NO: 49 - protein, 165 aa, synthetic construct
  REGION 1..165: note = synthetic peptide construct
MWLQSLLLLGTVACSISQGQMVHQAISPRTLNAWVKVLAKEEKAFSPEVIPMFSALSEGATPQDLNAAKVGGHQAAMQMLKETINEEAAEWDRAAAEPRGSDIAGTTSTLQEQIGWAAAKRWIILGLNKIVRMYSPTSIAAKYVDRFYKTLRAEQADYKDDDDKL

SEQ ID NO: 50 - protein, 20 aa, synthetic construct
  REGION 1..20: note = synthetic peptide construct
QGQMVHQAISPRTLNAWVKV

SEQ ID NO: 51 - protein, 26 aa, synthetic construct
  REGION 1..26: note = synthetic peptide construct
EEKAFSPEVIPMFSALSEGATPQDLN

SEQ ID NO: 52 - protein, 156 aa, synthetic construct
  REGION 1..156: note = synthetic peptide construct
MWLQSLLLLGTVACSISQGQMVHQALSPRTLNAWVKVLAKEEKGFNPEVIPMFTALSEGATPQDLNAAKVGGHQAAMQMLKDTINEEAAEWDRAAAEPRGSDIAGTTSTLQEQIAWAAAKRWIILGLNKIVRMYSPVSIAAKYVDRFFKTLRAEQA

SEQ ID NO: 53 - protein, 155 aa, synthetic construct
  REGION 1..155: note = synthetic peptide construct
MWLQSLLLLGTVACSISEEKGFNPEVIPMFTALSEGATPQDLNAAKVGGHQAAMQMLKDTINEEAAEWDRAAAEPRGSDIAGTTSTLQEQIAWAAAKRWIILGLNKIVRMYSPVSIAAKYVDRFFKTLRAEQAALQGQMVHQALSPRTLNAWVKV

SEQ ID NO: 54 - protein, 155 aa, synthetic construct
  REGION 1..155: note = synthetic peptide construct
MWLQSLLLLGTVACSISEEKAFSPEVIPMFSALSEGATPQDLNAAKVGGHQAAMQMLKETINEEAAEWDRAAAEPRGSDIAGTTSTLQEQIGWAAAKRWIILGLNKIVRMYSPTSIAAKYVDRFYKTLRAEQAALQGQMVHQAISPRTLNAWVKV

SEQ ID NO: 55 - protein, 20 aa, synthetic construct
  REGION 1..20: note = synthetic peptide construct
QGQMVHQALSPRTLNAWVKV

SEQ ID NO: 56 - protein, 26 aa, synthetic construct
  REGION 1..26: note = synthetic peptide construct
EEKGFNPEVIPMFTALSEGATPQDLN

SEQ ID NO: 57 - protein, 14 aa, synthetic construct
  REGION 1..14: note = synthetic peptide construct
QPISPRTLNAWVKV

SEQ ID NO: 58 - protein, 14 aa, synthetic construct
  REGION 1..14: note = synthetic peptide construct
QALSPRTLNAWVKV

SEQ ID NO: 59 - protein, 30 aa, synthetic construct
  REGION 1..30: note = synthetic peptide construct
EEKAFSPEVIPMFSALSEGATPQDLNTMLN

SEQ ID NO: 60 - protein, 30 aa, synthetic construct
  REGION 1..30: note = synthetic peptide construct
EEKGFNPEVIPMFTALSEGATPQDLNMMLN

SEQ ID NO: 61 - protein, 21 aa, synthetic construct
  REGION 1..21: note = synthetic peptide construct
PRGSDIAGTTSTLQEQIGWMT

SEQ ID NO: 62 - protein, 21 aa, synthetic construct
  REGION 1..21: note = synthetic peptide construct
PRGSDIAGTTSTLQEQIAWMT

SEQ ID NO: 63 - protein, 20 aa, synthetic construct
  REGION 1..20: note = synthetic peptide construct
SILDIRQGPKEPFRDYVDRF

SEQ ID NO: 64 - protein, 20 aa, synthetic construct
  REGION 1..20: note = synthetic peptide construct
SILDIKQGPKEPFRDYVDRF

SEQ ID NO: 65 - protein, 15 aa, synthetic construct
  REGION 1..15: note = synthetic peptide construct
QNSNPDCKTILKALG

SEQ ID NO: 66 - protein, 15 aa, synthetic construct
  REGION 1..15: note = synthetic peptide construct
QNANPDCKTILKALG

SEQ ID NO: 67 - protein, 25 aa, synthetic construct
  REGION 1..25: note = synthetic peptide construct
LEEMMTACQGVGGPGHKARILAEAM

SEQ ID NO: 68 - protein, 25 aa, synthetic construct
  REGION 1..25: note = synthetic peptide construct
LEEMMTACQGVGGPSHKARVLAEAM

SEQ ID NO: 69 - protein, 401 aa, synthetic construct
  REGION 1..401: note = synthetic peptide construct
MRVTEIRKSYQHWWRWGIMLLGILMICNAEEKLWVTVYYGVPVWKEATTTLFCASDRKAYDTEVHNVWATHACVPTDPNPQEVELKNVTENFNMWKNNMVEQMHEDIISLWDQSLKPCVKLTPLCVTLNCTDLRNATNGNDTNTTSSSRGMVGGGEMKNCSFNITTNIRGKVQKEYALFYKLDIAPIDNNSNNRYRLISCGAKFEPIPIHYCTPAGFAGAKVQCTHGIRPVVSTQLLLNGSLAEAADSGGDPEIVMHSFNCGGEFFYCGAKDNWRSELYKYKVVAAKARRRVVQREKRAGAVGFLGTAGSTMGAASVAVLTVQARLLLSGIVQQQNNLLRAIEAQQHLLQLTVWGIKQLQARAADWLWYIKIFIMIVGGLVGLRIAAFRVRKGYSPLSLQT

SEQ ID NO: 70 - protein, 17 aa, synthetic construct
  REGION 1..17: note = synthetic peptide construct
PIPIHYCAPAGFAILKC

SEQ ID NO: 71 - protein, 17 aa, synthetic construct
  REGION 1..17: note = synthetic peptide construct
PIPIHYCTPAGYAILKC

SEQ ID NO: 72 - protein, 27 aa, synthetic construct
  REGION 1..27: note = synthetic peptide construct
NVSTVQCTHGIRPVVSTQLLLNGSLAE

SEQ ID NO: 73 - protein, 27 aa, synthetic construct
  REGION 1..27: note = synthetic peptide construct
NVSSVQCTHGIKPVVSTQLLLNGSLAE

SEQ ID NO: 74 - protein, 20 aa, synthetic construct
  REGION 1..20: note = synthetic peptide construct
GGDPEIVMHTFNCGGEFFYC

SEQ ID NO: 75 - protein, 20 aa, synthetic construct
  REGION 1..20: note = synthetic peptide construct
GGDLEITTHSFNCRGEFFYC

SEQ ID NO: 76 - protein, 11 aa, synthetic construct
  REGION 1..11: note = synthetic peptide construct
CRIKQIINMWQ

SEQ ID NO: 77 - protein, 11 aa, synthetic construct
  REGION 1..11: note = synthetic peptide construct
CKIRQIVNRWQ

SEQ ID NO: 78 - protein, 18 aa, synthetic construct
  REGION 1..18: note = synthetic peptide construct
GGDMRDNWRSELYKYKVV

SEQ ID NO: 79 - protein, 18 aa, synthetic construct
  REGION 1..18: note = synthetic peptide construct
GGNMKDNWRSELYKYKVV

SEQ ID NO: 80 - protein, 46 aa, synthetic construct
  REGION 1..46: note = synthetic peptide construct
LTVQARLLLSGIVQQQNNLLRAIEAQQHLLQLTVWGIKQLQARVLA

SEQ ID NO: 81 - protein, 46 aa, synthetic construct
  REGION 1..46: note = synthetic peptide construct
LTVQARQLLSGIVQQQSNLLKAIEAQQHMLQLTVWGIKQLQTRVLA

SEQ ID NO: 82 - protein, 16 aa, synthetic construct
  REGION 1..16: note = synthetic peptide construct
DQQLLGIWGCSGKLIC

SEQ ID NO: 83 - protein, 16 aa, synthetic construct
  REGION 1..16: note = synthetic peptide construct
DQQLLGLWGCSGKLIC

SEQ ID NO: 84 - protein, 20 aa, synthetic construct
  REGION 1..20: note = synthetic peptide construct
WLWYIKIFIMIVGGLVGLRI

SEQ ID NO: 85 - protein, 20 aa, synthetic construct
  REGION 1..20: note = synthetic peptide construct
WLWYIRIFIMIVGGLIGLRI

SEQ ID NO: 86 - protein, 4 aa, synthetic construct
  REGION 1..4: note = synthetic peptide construct
AAAE

SEQ ID NO: 87 - protein, 4 aa, synthetic construct
  REGION 1..4: note = synthetic peptide construct
AAAA

SEQ ID NO: 88 - protein, 5 aa, synthetic construct
  REGION 1..5: note = synthetic peptide construct
AAAAL

SEQ ID NO: 89 - DNA, 1209 bp, synthetic construct
  misc_feature 1..1209: note = synthetic nucleotide sequence Env-CE1_V1V2 BaL
  source 1..1209: mol_type = other DNA
atgcgggtgacggagatccggaagtcgtatcagcactggtggcggtggggcatcatgctccttgggatactgatgatctgcaacgccgaggagaagctgtgggtcacggtgtactacggggtcccggtctggaaggaggccaccacgaccctgttctgcgcgagcgaccgcaaggcctacgacaccgaggtgcacaacgtgtgggctacgcacgcgtgcgtgccaacggaccctaacccgcaggaggtggaactgaagaacgtgaccgagaacttcaacatgtggaagaacaacatggtggagcagatgcacgaggacatcatctccctgtgggaccagtcgctgaagccgtgcgtcaagctgacgccgctctgcgtcacgctgaactgcaccgacctgcgcaacgccacgaacggcaacgacaccaacaccactagtagctcgcgcggcatggtgggcggcggcgagatgaagaactgcagcttcaacatcacgaccaacatccgcggcaaggtgcagaaggagtacgccctgttctacaagctggacatcgcccctatcgacaacaacagcaacaaccgctaccggctgatcagctgcggcgctaagttcgagccgatccctatccactactgcacgccagctggattcgcgggagcgaaggtgcagtgcacgcacggcatccgacctgtggtctcgacgcagctgctcctgaacggaagcctggcagaggcagctgacagcggcggggacccggagatcgtcatgcactccttcaactgcgggggcgagttcttctactgcggagccaaggacaactggcggtctgagctgtacaagtacaaggtcgtggctgcgaaggcgcgacggagggtggtccagcgcgagaagcgagccggtgcagtgggcttccttgggacggccggctcgacgatgggagcggcatcggtcgcggtgctgacggtccaggcgaggctgctgctcagcgggatcgtccagcagcagaacaacctgctccgggcgatcgaggcgcagcagcacctgctccagttaacggtctggggcatcaagcagctgcaggctcgagccgcggactggctctggtacatcaagatcttcatcatgatcgtgggcggactggtcggcctgcgaatcgctgcattccgcgtccggaaggggtactcgcctctcagcctccaaacgtgataa